European Patent Application EP 4 372 101 A1, published May 22, 2024. Title: METHODS AND DEVICES OF GENERATING CLUSTERS OF AMPLICONS. Applicant: ESBIOLAB LLC. The sequence listing filed with the application follows.

SEQUENCE LISTING (7 sequences)

SEQ ID NO: 1 - DNA, 24 bp, synthetic construct
  source 1..24: mol_type = other DNA
caagcagaagacggcatacgagat

SEQ ID NO: 2 - DNA, 29 bp, synthetic construct
  source 1..29: mol_type = other DNA
  misc_feature 1..5: note = DNA
  misc_feature 6: note = RNA
  misc_feature 7..29: note = DNA
aatgatacggcgaccaccgagatctacac

SEQ ID NO: 3 - DNA, 44 bp, synthetic construct
  source 1..44: mol_type = other DNA
aaaaaaaaaaaaaaaaaaaacaagcagaagacggcatacgagat

SEQ ID NO: 4 - DNA, 39 bp, synthetic construct
  source 1..39: mol_type = other DNA
  misc_feature 1..15: note = DNA
  misc_feature 16: note = RNA
  misc_feature 17..39: note = DNA
ttttttttttaatgatacggcgaccaccgagatctacac

SEQ ID NO: 5 - DNA, 47 bp, synthetic construct
  source 1..47: mol_type = other DNA
  modified_base 10: mod_base = OTHER; note = 5-Octadiynyl uracil
  misc_feature 1..23: note = DNA
  misc_feature 24: note = RNA
  misc_feature 25..47: note = DNA
tttttttttnttttttttaatgatacggcgaccaccgagatctacac

SEQ ID NO: 6 - RNA, 20 nt, synthetic construct
  source 1..20: mol_type = other RNA
aaaaaaaaaaaaaaaaaaaa

SEQ ID NO: 7 - DNA, 25 bp, synthetic construct
  source 1..25: mol_type = other DNA
ttttttttttttttttttttttttt